European Patent Specification EP 3 980 411 B1, published July 23, 2025. Title: COMPOUNDS. Applicant: Step Pharma S.A.S. The sequence listing filed with the application follows.

SEQUENCE LISTING (2 sequences)

SEQ ID NO: 1 - protein, 20 aa, Artificial Sequence
  synthetic
GGDYKDDDDKGGHHHHHHHH

SEQ ID NO: 2 - protein, 29 aa, Artificial Sequence
  synthetic
DYKDDDDKHHHHHHGLNDIFEAQKIEWHE